European Patent Application EP 4 692 106 A1, published February 11, 2026. Title: PEPTIDE PROMOTING HAIR HAIR GROWTH OR INHIBITING HAIR LOSS AND USES THEREOF. Applicant: CAREGEN CO., LTD. Application WO. The sequence listing filed with the application follows.

SEQUENCE LISTING (10 sequences)

SEQ ID NO: 1 - protein, 10 aa, synthetic construct
AERRREKCRC

SEQ ID NO: 2 - DNA, 20 bp, synthetic construct
  source 1..20: mol_type = other DNA
ccagctattgtaacacctca

SEQ ID NO: 3 - DNA, 20 bp, synthetic construct
  source 1..20: mol_type = other DNA
ttcagatgtaggcagctgtc

SEQ ID NO: 4 - DNA, 25 bp, synthetic construct
  source 1..25: mol_type = other DNA
accagcagcgactctgaggaggaac

SEQ ID NO: 5 - DNA, 26 bp, synthetic construct
  source 1..26: mol_type = other DNA
tgaccctcttggcagcaggatagtcc

SEQ ID NO: 6 - DNA, 28 bp, synthetic construct
  source 1..28: mol_type = other DNA
accttcgttgccctctgtgccacagatg

SEQ ID NO: 7 - DNA, 21 bp, synthetic construct
  source 1..21: mol_type = other DNA
aggcccggaggcagtccgggt

SEQ ID NO: 8 - DNA, 20 bp, synthetic construct
  source 1..20: mol_type = other DNA
ggagccaaaagggtcatcat

SEQ ID NO: 9 - DNA, 20 bp, synthetic construct
  source 1..20: mol_type = other DNA
gtgatggcatggactgtggt

SEQ ID NO: 10 - protein, 10 aa, synthetic construct
AERRRELCRC